European Patent Specification EP 3 790 931 B1, published September 27, 2023. Title: Sulforhodamine Phosphoramidite Dyes. Applicant: Cepheid Lund, Kevin P. Sergueev, Dmitri Qabar, Maher N. Gall, Alexander. The sequence listing filed with the application follows.

SEQUENCE LISTING (7 sequences)

SEQ ID NO: 1 - DNA, 17 bp, Synthetic
tcagagtacctgaaaca

SEQ ID NO: 2 - DNA, 23 bp, Synthetic
  misc_feature (3)..(3): 2,6-diaminopurine
  misc_feature (7)..(7): 2,6-diaminopurine
  misc_feature (11)..(11): 2,6-diaminopurine
  misc_feature (15)..(15): 2,6-diaminopurine
ccncggngcgngacntctcggcc

SEQ ID NO: 3 - DNA, 20 bp, Synthetic
  misc_feature (3)..(3): 2,6-diaminopurine
  misc_feature (5)..(5): 2,6-diaminopurine
  misc_feature (20)..(20): 2,6-diaminopurine
ccngngcaaactgggcggcn

SEQ ID NO: 4 - DNA, 27 bp, Synthetic
aaacctccaggccagaaagagagagta

SEQ ID NO: 5 - DNA, 29 bp, Synthetic
aaaaggcattcctgaagctgacagcattc

SEQ ID NO: 6 - DNA, 26 bp, Synthetic
aaaacctgccttctgcgtgagattct

SEQ ID NO: 7 - DNA, 26 bp, Synthetic
ctgtacgaaaagaccacagggcccat